European Patent Specification EP 3 915 553 B1, published March 26, 2025. Title: Compositions comprising amino acids for use in the treatment of mitochondrial dysfunction-related diseases. Applicant: Professional Dietetics S.p.A. et al. The sequence listing filed with the application follows.

SEQUENCE LISTING (16 sequences)

SEQ ID NO: 1 - DNA, 20 bp, Artificial Sequence
  GAPDH Primer sense 5'-3'
aactttggcattgtggaagg

SEQ ID NO: 2 - DNA, 20 bp, Artificial Sequence
  GAPDH Primer Antisense 5'-3'
acacattgggggtaggaaca

SEQ ID NO: 3 - DNA, 22 bp, Artificial Sequence
  Primer Cyt c Sense 5'-3'
ataggggcatgtcacctcaaac

SEQ ID NO: 4 - DNA, 22 bp, Artificial Sequence
  Primer Cyt c Antisense 5'-3'
gtggttagccatgacctgaaag

SEQ ID NO: 5 - DNA, 24 bp, Artificial Sequence
  Primer PGC-1a Sense 5'-3'
actatgaatcaagccactacagac

SEQ ID NO: 6 - DNA, 22 bp, Artificial Sequence
  Primer PGC-1a Antisense 5'-3'
ttcatccctcttgagcctttcg

SEQ ID NO: 7 - DNA, 25 bp, Artificial Sequence
  Primer Tfam Sense 5'-3'
aagacctcgttcagcatataacatt

SEQ ID NO: 8 - DNA, 23 bp, Artificial Sequence
  Primer Tfam Antisense 5'-3'
ttttccaagcctcatttacaagc

SEQ ID NO: 9 - DNA, 21 bp, Artificial Sequence
  Primer KFL15 Sense 5'-3'
acaccaagagcagccacctca

SEQ ID NO: 10 - DNA, 20 bp, Artificial Sequence
  Primer KFL15 Antisense 5'-3'
tgagatcgccggtgccttga

SEQ ID NO: 11 - DNA, 18 bp, Artificial Sequence
  Primer PP2CM Sense 5'-3'
accacaggcaggcgactc

SEQ ID NO: 12 - DNA, 22 bp, Artificial Sequence
  Primer PP2CM Antisense 5'-3'
tggctcatcaatgcggttatcc

SEQ ID NO: 13 - DNA, 23 bp, Artificial Sequence
  Primer mtDNA Sense 5'-3'
acatgcaaacctccatagaccgg

SEQ ID NO: 14 - DNA, 20 bp, Artificial Sequence
  Primer mtDNA Antisense 5'-3'
tcactgctgagtcccgtggg

SEQ ID NO: 15 - DNA, 20 bp, Artificial Sequence
  Primer gDNA Sense 5'-3'
ggtcgcggtgtgggcatttg

SEQ ID NO: 16 - DNA, 20 bp, Artificial Sequence
  Primer gDNA Antisense 5'-3'
cgtgatcgtagcgtctggtt